European Patent Application EP 4 342 978 A2, published March 27, 2024. Title: Gold Optimized CAR T-cells. Applicant: Chimera Bioengineering, Inc. Application EP. The sequence listing filed with the application follows.

SEQUENCE LISTING (32 sequences)

SEQ ID NO: 1 - RNA, 98 nt, synthetic construct
  source 1..98: mol_type = other RNA
gcgcgtcctggattaaaacataccagatttcgatctggagaggtgaagaatacgaccacctaatccagctgatgagtcccaaataggacgaaacgcgc

SEQ ID NO: 2 - RNA, 110 nt, synthetic construct
  source 1..110: mol_type = other RNA
gcgcgtcctggattcnnnnntaaaacataccagatttcggtctggagaggtgaagaatacgaccacctannnnnatccagctgatgagtcccaaataggacgaaacgcgc

SEQ ID NO: 3 - RNA, 31 nt, synthetic construct
  source 1..31: mol_type = other RNA
acgtcgacttatattgcatggttcgtgacgt

SEQ ID NO: 4 - RNA, 37 nt, synthetic construct
  source 1..37: mol_type = other RNA
cgaaccggccttatattgcatggtgcgttgcggctcg

SEQ ID NO: 5 - RNA, 66 nt, synthetic construct
  source 1..66: mol_type = other RNA
gctgtcaccggatgcttggtacgttatattcagtccggtctgatgagtccgtgaggacgaaacagc

SEQ ID NO: 6 - RNA, 76 nt, synthetic construct
  source 1..76: mol_type = other RNA
gctgtcaccggatggcgttgcgtggtacgttatattccggccatctggtctgatgagtccgtgaggacgaaacagc

SEQ ID NO: 7 - RNA, 67 nt, synthetic construct
  source 1..67: mol_type = other RNA
gctgtcaccggattgcgtggtacgttatattccgtccggtctgatgagtccgtgaggacgaaacagc

SEQ ID NO: 8 - skipped

SEQ ID NO: 9 - RNA, 13 nt, synthetic construct
  source 1..13: mol_type = other RNA
atttatttattta

SEQ ID NO: 10-23 - skipped (14 entries)

SEQ ID NO: 24 - protein, 18 aa, Thoseaasigna virus 2A
EGRGSLLTCGDVEENPGP

SEQ ID NO: 25 - protein, 19 aa, Porcine teschovirus-1
ATNFSLLKQAGDVEENPGP

SEQ ID NO: 26 - protein, 20 aa, Equine rhinitis A virus
QCTNYALLKLAGDVESNPGP

SEQ ID NO: 27 - protein, 22 aa, Foot-and-mouth disease virus
VKQTLNFDLLKLAGDVESNPGP

SEQ ID NO: 28 - DNA, 282 bp, Homo sapiens
  source 1..282: mol_type = genomic DNA
taattaagtgcttcccacttaaaacatatcaggccttctatttatttaaatatttaaattttatatttattgttgaatgtatggtttgctacctattgtaactattattcttaatcttaaaactataaatatggatcttttatgattctttttgtaagccctaggggctctaaaatggtttcacttatttatcccaaaatatttattattatgttgaatgttaaatatagtatctatgtagattggttagtaaaactatttaataaatttgataaatataaa

SEQ ID NO: 29 - DNA, 282 bp, Homo sapiens
  source 1..282: mol_type = genomic DNA
taattaagtgcttcccacttaaaacatatcaggccttctatttatttaaatatttaaattttatatttattgttgaatgtatggtttgctacctattgtaactattattcttaatcttaaaactataaatatggatcttttatgattgaatttgtaagccctaggggctctaaaatggtttcacttatttatcccaaaatatttattattatgttgaatgttaaatatagtatctatgtagattggttagtaaaactatttaataaatttgataaatataaa

SEQ ID NO: 30 - DNA, 585 bp, Homo sapiens
  source 1..585: mol_type = genomic DNA
tggttgtcctgcctgcaatatttgaattttaaatctaaatctatttattaatatttaacattatttatatggggaatatatttttagactcatcaatcaaataagtatttataatagcaacttttgtgtaatgaaaatgaatatctattaatatatgtattatttataattcctatatcctgtgactgtctcacttaatcctttgttttctgactaattaggcaaggctatgtgattacaaggctttatctcaggggccaactaggcagccaacctaagcaagatcccatgggttgtgtgtttatttcacttgatgatacaatgaacacttataagtgaagtgatactatccagttactgccggtttgaaaatatgcctgcaatctgagccagtgctttaatggcatgtcagacagaacttgaatgtgtcaggtgaccctgatgaaaacatagcatctcaggagatttcatgcctggtgcttccaaatattgttgacaactgtgactgtacccaaatggaaagtaactcatttgttaaaattatcaatatctaatatatatgaataaagtgtaagttcacaacta

SEQ ID NO: 31 - DNA, 32 bp, synthetic construct
  source 1..32: mol_type = other DNA
tagagggtatataatggaagctcgacttccag

SEQ ID NO: 32 - DNA, 131 bp, synthetic construct
  source 1..131: mol_type = other DNA
ggaggaaaaactgtttcatacagaaggcgtggaggaaaaactgtttcatacagaaggcgtggaggaaaaactgtttcatacagaaggcgtagatctagactctagagggtatataatggaagctcgaattc